European Patent Application EP 4 310 195 A1, published January 24, 2024. Title: METHOD FOR NUCLEIC ACID DETECTION USING SIGNAL-MEDIATED AMPLIFICATION OF RNA TECHNOLOGY AND RNA APTAMERS. Applicant: Moirai Biodesign, S.L. The sequence listing filed with the application follows.

SEQUENCE LISTING (76 sequences)

SEQ ID NO: 1 - DNA, 34 bp, synthetic construct
  misc_feature 1..34: note = > E.coli 23S rRNA SMART-first probe and Fig. 4
  source 1..34: mol_type = other DNA
gcatttagctaccgggcagtgccattttcgaaat

SEQ ID NO: 2 - DNA, 102 bp, synthetic construct
  misc_feature 1..102: note = > E.coli 23S rRNA SMART-Mango second probe and Fig. 4
  misc_feature 75: note = /note="n = iSp18"
  misc_feature 102: note = /note="n=3amo"
  source 1..102: mol_type = other DNA
ggcacgtacgaatataccacataccaaaccttccttcgtacgtgccccctatagtgagtcgtattaatttcgaanggcatgacaacccgaacaccagtgatn

SEQ ID NO: 3 - RNA, 45 nt, synthetic construct
  misc_feature 1..45: note = > Mango-III (A10U) RNA aptamer
  source 1..45: mol_type = other RNA
ggcacgtacgaaggaaggtttgtatgtggtatattcgtacgtgcc

SEQ ID NO: 4 - DNA, 20 bp, synthetic construct
  misc_feature 1..20: note = > 5 primer for E.coli 16S rRNA NASBA amplification reaction
  source 1..20: mol_type = other DNA
ggaggcagcagtggggaata

SEQ ID NO: 5 - DNA, 45 bp, synthetic construct
  misc_feature 1..45: note = 3 primer for E.coli 16S rRNA NASBA amplification reaction
  source 1..45: mol_type = other DNA
aattctaatacgactcactatagggattaccgcggctgctggcac

SEQ ID NO: 6 - RNA, 1450 nt, synthetic construct
  misc_feature 1..1450: note = > NR 024570.1 Escherichia coli strain U 5/41 16S ribosomal RNA,partial sequence
  source 1..1450: mol_type = other RNA
agtttgatcatggctcagattgaacgctggcggcaggcctaacacatgcaagtcgaacggtaacaggaagcagcttgctgctttgctgacgagtggcggacgggtgagtaatgtctgggaaactgcctgatggagggggataactactggaaacggtagctaataccgcataacgtcgcaagcacaaagagggggaccttagggcctcttgccatcggatgtgcccagatgggattagctagtaggtggggtaacggctcacctaggcgacgatccctagctggtctgagaggatgaccagcaacactggaactgagacacggtccagactcctacgggaggcagcagtggggaatattgcacaatgggcgcaagcctgatgcagccatgcngcgtgtatgaagaaggccttcgggttgtaaagtactttcagcggggaggaagggagtaaagttaatacctttgctcattgacgttacccgcagaagaagcaccggctaactccgtgccagcagccgcggtaatacggagggtgcaagcgttaatcggaattactgggcgtaaagcgcacgcaggcggtttgttaagtcagatgtgaaatccccgggctcaacctgggaactgcatctgatactggcaagcttgagtctcgtagaggggggtagaattccaggtgtagcggtgaaatgcgtagagatctggaggaataccggtggcgaaggcggccccctggacgaagactgacgctcaggtgcgaaagcgtggggagcaaacaggattagataccctggtagtccacgccgtaaacgatgtcgacttggaggttgtgcccttgaggcgtggcttccgganntaacgcgttaagtcgaccgcctggggagtacggccgcaaggttaaaactcaaatgaattgacgggggccgcacaagcggtggagcatgtggtttaattcgatgcaacgcgaagaaccttacctggtcttgacatccacggaagttttcagagatgagaatgtgccttcgggaaccgtgagacaggtgctgcatggctgtcgtcagctcgtgttgtgaaatgttgggttaagtcccgcaacgagcgcaacccttatcctttgttgccagcggtccggccgggaactcaaaggagactgccagtgataaactggaggaaggtggggatgacgtcaagtcatcatggcccttacgaccagggctacacacgtgctacaatggcgcatacaaagagaagcgacctcgcgagagcaagcggacctcataaagtgcgtcgtagtccggattggagtctgcaactcgactccatgaagtcggaatcgctagtaatcgtggatcagaatgccacggtgaatacgttcccgggccttgtacacaccgcccgtcacaccatgggagtgggttgcaaaagaagtaggtagcttaacttcgggagggcg

SEQ ID NO: 7 - DNA, 37 bp, synthetic construct
  misc_feature 1..37: note = > E.coli 16S rRNA SMART-first probe (29-nt hybridization)
  source 1..37: mol_type = other DNA
tgatgcagccatgcggcgtgtatgaagaattcgaaat

SEQ ID NO: 8 - DNA, 105 bp, synthetic construct
  misc_feature 1..105: note = > E.coli 16S rRNA SMART-Mango second probe (29-nt hybridization)
  misc_feature 75: note = /note="n = iSp18"
  misc_feature 105: note = /note="n=3amo"
  source 1..105: mol_type = other DNA
ggcacgtacgaatataccacataccaaaccttccttcgtacgtgccccctatagtgagtcgtattaatttcgaanggccttcgggttgtaaagtactttcagcgn

SEQ ID NO: 9 - RNA, 191 nt, synthetic construct
  misc_feature 1..191: note = > Reverse Complement RNA sequence of E.coli 16S, NASBA product
  source 1..191: mol_type = other RNA
gggattaccgcggctgctggcacggagttagccggtgcttcttctgcgggtaacgtcaatgagcaaaggtattaactttactcccttcctccccgctgaaagtactttacaacccgaaggccttcttcatacacgccgcatggctgcatcaggcttgcgcccattgtgcaatattccccactgctgcctcc

SEQ ID NO: 10 - DNA, 31 bp, synthetic construct
  misc_feature 1..31: note = > E.coli 16S rRNA SMART-first probe, 2-complementary (3WJ)nucleotides
  source 1..31: mol_type = other DNA
tgatgcagccatgcggcgtgtatgaagaatt

SEQ ID NO: 11 - DNA, 33 bp, synthetic construct
  misc_feature 1..33: note = > E.coli 16S rRNA SMART-first probe, 4-complementary (3WJ)nucleotides
  source 1..33: mol_type = other DNA
tgatgcagccatgcggcgtgtatgaagaattcg

SEQ ID NO: 12 - DNA, 35 bp, synthetic construct
  misc_feature 1..35: note = > E.coli 16S rRNA SMART-first probe, 6-complementary (3WJ)nucleotides
  source 1..35: mol_type = other DNA
tgatgcagccatgcggcgtgtatgaagaattcgaa

SEQ ID NO: 13 - RNA, 75 nt, synthetic construct
  misc_feature 1..75: note = > Synthetic RNA target of E.coli 16S ribosomal RNA (75-nt, pos.357-432, reverse complement)
  source 1..75: mol_type = other RNA
tgaaagtactttacaacccgaaggccttcttcatacacgcggcatggctgcatcaggcttgcgcccattgtgcaa

SEQ ID NO: 14 - DNA, 39 bp, synthetic construct
  misc_feature 1..39: note = > E.coli 16S rRNA SMART-first probe, 10-complementary (3WJ)nucleotides
  source 1..39: mol_type = other DNA
tgatgcagccatgcggcgtgtatgaagaattcgaaatta

SEQ ID NO: 15 - DNA, 44 bp, synthetic construct
  misc_feature 1..44: note = > E.coli 16S rRNA SMART-first probe, 15-complementary (3WJ)nucleotides
  source 1..44: mol_type = other DNA
tgatgcagccatgcggcgtgtatgaagaattcgaaattaatacg

SEQ ID NO: 16 - DNA, 36 bp, synthetic construct
  misc_feature 1..36: note = > E.coli 16S rRNA SMART-first probe, 1-nt of separation from thesecond-probe hybridization region
  source 1..36: mol_type = other DNA
tgatgcagccatgcggcgtgtatgaagattcgaaat

SEQ ID NO: 17 - DNA, 35 bp, synthetic construct
  misc_feature 1..35: note = > E.coli 16S rRNA SMART-first probe, 2-nt of separation from thesecond-probe hybridization region
  source 1..35: mol_type = other DNA
tgatgcagccatgcggcgtgtatgaagttcgaaat

SEQ ID NO: 18 - DNA, 33 bp, synthetic construct
  misc_feature 1..33: note = > E.coli 16S rRNA SMART-first probe, 4-nt of separation from thesecond-probe hybridization region
  source 1..33: mol_type = other DNA
tgatgcagccatgcggcgtgtatgattcgaaat

SEQ ID NO: 19 - DNA, 31 bp, synthetic construct
  misc_feature 1..31: note = > E.coli 16S rRNA SMART-first probe, 6-nt of separation from thesecond-probe hybridization region
  source 1..31: mol_type = other DNA
tgatgcagccatgcggcgtgtatttcgaaat

SEQ ID NO: 20 - DNA, 30 bp, synthetic construct
  misc_feature 1..30: note = > E.coli 16S rRNA SMART-first probe (22-nt hybridization)
  source 1..30: mol_type = other DNA
gccatgcggcgtgtatgaagaattcgaaat

SEQ ID NO: 21 - DNA, 23 bp, synthetic construct
  misc_feature 1..23: note = > E.coli 16S rRNA SMART-first probe (15-nt hybridization)
  source 1..23: mol_type = other DNA
ggcgtgtatgaagaattcgaaat

SEQ ID NO: 22 - DNA, 15 bp, synthetic construct
  misc_feature 1..15: note = > E.coli 16S rRNA SMART-first probe (7-nt hybridization)
  source 1..15: mol_type = other DNA
tgaagaattcgaaat

SEQ ID NO: 23 - DNA, 98 bp, synthetic construct
  misc_feature 1..98: note = > E.coli 16S rRNA SMART-Mango second probe (22-nt hybridization)
  misc_feature 75: note = /note="n = iSp18"
  misc_feature 98: note = /note="n=3amo"
  source 1..98: mol_type = other DNA
ggcacgtacgaatataccacataccaaaccttccttcgtacgtgccccctatagtgagtcgtattaatttcgaanggccttcgggttgtaaagtactn

SEQ ID NO: 24 - DNA, 91 bp, synthetic construct
  misc_feature 1..91: note = > E.coli 16S rRNA SMART-Mango second probe (15-nt hybridization)
  misc_feature 75: note = /note="n = iSp18"
  misc_feature 91: note = /note="n=3amo"
  source 1..91: mol_type = other DNA
ggcacgtacgaatataccacataccaaaccttccttcgtacgtgccccctatagtgagtcgtattaatttcgaanggccttcgggttgtan

SEQ ID NO: 25 - DNA, 83 bp, synthetic construct
  misc_feature 1..83: note = > E.coli 16S rRNA SMART-Mango second probe (7-nt hybridization)
  misc_feature 75: note = /note="n = iSp18"
  misc_feature 83: note = /note="n=3amo"
  source 1..83: mol_type = other DNA
ggcacgtacgaatataccacataccaaaccttccttcgtacgtgccccctatagtgagtcgtattaatttcgaanggccttcn

SEQ ID NO: 26 - DNA, 38 bp, synthetic construct
  misc_feature 1..38: note = > SARS-CoV-2 T3 SMART-first probe
  source 1..38: mol_type = other DNA
ttggttccatgctatacatgtctctgggacttcgaaat

SEQ ID NO: 27 - DNA, 106 bp, synthetic construct
  misc_feature 1..106: note = > SARS-CoV-2 T3 SMART-Mango second probe
  misc_feature 75: note = /note="n = iSp18"
  misc_feature 106: note = /note="n=3amo"
  source 1..106: mol_type = other DNA
ggcacgtacgaatataccacataccaaaccttccttcgtacgtgccccctatagtgagtcgtattaatttcgaancaatggtactaagaggtttgataaccctgtn

SEQ ID NO: 28 - RNA, 30 nt, synthetic construct
  misc_feature 1..30: note = > Synthetic RNA target of SARS-CoV-2 S spike RNA (30-nt, pos.21766-21795, reverse complement)
  source 1..30: mol_type = other RNA
ctcttagtaccattggtcccagagacatgt

SEQ ID NO: 29 - RNA, 189 nt, synthetic construct
  misc_feature 1..189: note = > Reverse Complement RNA sequence of SARS-CoV-2 product of NASBA(189-
  source 1..189: mol_type = other RNA
cagtggaagcaaaataaacaccatcattaaatggtaggacagggttatcaaacctcttagtaccattggtcccagagacatgtatagcatggaaccaagtaacattggaaaagaaaggtaagaacaagtcctgagttgaatgtaaaactgaggatctgaaaactttgtcagggtaataaacaccacgtg

SEQ ID NO: 30 - DNA, 85 bp, synthetic construct
  misc_feature 1..85: note = > SARS-CoV-2 T3 SMART- second probe for Molecular Beacondetection
  misc_feature 54: note = /note="n = iSp18"
  misc_feature 85: note = /note="n=3amo"
  source 1..85: mol_type = other DNA
tgaagaaggccttcgggttgtaaagccctatagtgagtcgtattaatttcgaancaatggtactaagaggtttgataaccctgtn

SEQ ID NO: 31 - DNA, 39 bp, synthetic construct
  misc_feature 1..39: note = > Molecular Beacon Oligonucleotide probe
  misc_feature 1: note = /note="n=5-6-FAM"
  misc_feature 39: note = /note="n=3-Dabcyl"
  source 1..39: mol_type = other DNA
ncgagcttgaagaaggccttcgggttgtaaagagctcgn

SEQ ID NO: 32 - RNA, 3822 nt, synthetic construct
  misc_feature 1..3822: note = > S spike surface glycoprotein RNA (CDS);NC_045512.2:21563-25384 Severe acute respiratory syndromecoronavirus 2 isolate Wuhan-Hu-1 (SARS-CoV-2), complete genome
  source 1..3822: mol_type = other RNA
atgtttgtttttcttgttttattgccactagtctctagtcagtgtgttaatcttacaaccagaactcaattaccccctgcatacactaattctttcacacgtggtgtttattaccctgacaaagttttcagatcctcagttttacattcaactcaggacttgttcttacctttcttttccaatgttacttggttccatgctatacatgtctctgggaccaatggtactaagaggtttgataaccctgtcctaccatttaatgatggtgtttattttgcttccactgagaagtctaacataataagaggctggatttttggtactactttagattcgaagacccagtccctacttattgttaataacgctactaatgttgttattaaagtctgtgaatttcaattttgtaatgatccatttttgggtgtttattaccacaaaaacaacaaaagttggatggaaagtgagttcagagtttattctagtgcgaataattgcacttttgaatatgtctctcagccttttcttatggaccttgaaggaaaacagggtaatttcaaaaatcttagggaatttgtgtttaagaatattgatggttattttaaaatatattctaagcacacgcctattaatttagtgcgtgatctccctcagggtttttcggctttagaaccattggtagatttgccaataggtattaacatcactaggtttcaaactttacttgctttacatagaagttatttgactcctggtgattcttcttcaggttggacagctggtgctgcagcttattatgtgggttatcttcaacctaggacttttctattaaaatataatgaaaatggaaccattacagatgctgtagactgtgcacttgaccctctctcagaaacaaagtgtacgttgaaatccttcactgtagaaaaaggaatctatcaaacttctaactttagagtccaaccaacagaatctattgttagatttcctaatattacaaacttgtgcccttttggtgaagtttttaacgccaccagatttgcatctgtttatgcttggaacaggaagagaatcagcaactgtgttgctgattattctgtcctatataattccgcatcattttccacttttaagtgttatggagtgtctcctactaaattaaatgatctctgctttactaatgtctatgcagattcatttgtaattagaggtgatgaagtcagacaaatcgctccagggcaaactggaaagattgctgattataattataaattaccagatgattttacaggctgcgttatagcttggaattctaacaatcttgattctaaggttggtggtaattataattacctgtatagattgtttaggaagtctaatctcaaaccttttgagagagatatttcaactgaaatctatcaggccggtagcacaccttgtaatggtgttgaaggttttaattgttactttcctttacaatcatatggtttccaacccactaatggtgttggttaccaaccatacagagtagtagtactttcttttgaacttctacatgcaccagcaactgtttgtggacctaaaaagtctactaatttggttaaaaacaaatgtgtcaatttcaacttcaatggtttaacaggcacaggtgttcttactgagtctaacaaaaagtttctgcctttccaacaatttggcagagacattgctgacactactgatgctgtccgtgatccacagacacttgagattcttgacattacaccatgttcttttggtggtgtcagtgttataacaccaggaacaaatacttctaaccaggttgctgttctttatcaggatgttaactgcacagaagtccctgttgctattcatgcagatcaacttactcctacttggcgtgtttattctacaggttctaatgtttttcaaacacgtgcaggctgtttaataggggctgaacatgtcaacaactcatatgagtgtgacatacccattggtgcaggtatatgcgctagttatcagactcagactaattctcctcggcgggcacgtagtgtagctagtcaatccatcattgcctacactatgtcacttggtgcagaaaattcagttgcttactctaataactctattgccatacccacaaattttactattagtgttaccacagaaattctaccagtgtctatgaccaagacatcagtagattgtacaatgtacatttgtggtgattcaactgaatgcagcaatcttttgttgcaatatggcagtttttgtacacaattaaaccgtgctttaactggaatagctgttgaacaagacaaaaacacccaagaagtttttgcacaagtcaaacaaatttacaaaacaccaccaattaaagattttggtggttttaatttttcacaaatattaccagatccatcaaaaccaagcaagaggtcatttattgaagatctacttttcaacaaagtgacacttgcagatgctggcttcatcaaacaatatggtgattgccttggtgatattgctgctagagacctcatttgtgcacaaaagtttaacggccttactgttttgccacctttgctcacagatgaaatgattgctcaatacacttctgcactgttagcgggtacaatcacttctggttggacctttggtgcaggtgctgcattacaaataccatttgctatgcaaatggcttataggtttaatggtattggagttacacagaatgttctctatgagaaccaaaaattgattgccaaccaatttaatagtgctattggcaaaattcaagactcactttcttccacagcaagtgcacttggaaaacttcaagatgtggtcaaccaaaatgcacaagctttaaacacgcttgttaaacaacttagctccaattttggtgcaatttcaagtgttttaaatgatatcctttcacgtcttgacaaagttgaggctgaagtgcaaattgataggttgatcacaggcagacttcaaagtttgcagacatatgtgactcaacaattaattagagctgcagaaatcagagcttctgctaatcttgctgctactaaaatgtcagagtgtgtacttggacaatcaaaaagagttgatttttgtggaaagggctatcatcttatgtccttccctcagtcagcacctcatggtgtagtcttcttgcatgtgacttatgtccctgcacaagaaaagaacttcacaactgctcctgccatttgtcatgatggaaaagcacactttcctcgtgaaggtgtctttgtttcaaatggcacacactggtttgtaacacaaaggaatttttatgaaccacaaatcattactacagacaacacatttgtgtctggtaactgtgatgttgtaataggaattgtcaacaacacagtttatgatcctttgcaacctgaattagactcattcaaggaggagttagataaatattttaagaatcatacatcaccagatgttgatttaggtgacatctctggcattaatgcttcagttgtaaacattcaaaaagaaattgaccgcctcaatgaggttgccaagaatttaaatgaatctctcatcgatctccaagaacttggaaagtatgagcagtatataaaatggccatggtacatttggctaggttttatagctggcttgattgccatagtaatggtgacaattatgctttgctgtatgaccagttgctgtagttgtctcaagggctgttgttcttgtggatcctgctgcaaatttgatgaagacgactctgagccagtgctcaaaggagtcaaattacattacacataa

SEQ ID NO: 33 - DNA, 24 bp, synthetic construct
  misc_feature 1..24: note = > 5 primer for SARS-CoV-2 NASBA amplification reaction
  source 1..24: mol_type = other DNA
cacgtggtgtttattaccctgaca

SEQ ID NO: 34 - DNA, 49 bp, synthetic construct
  misc_feature 1..49: note = > 3 primer for SARS-CoV-2 NASBA amplification reaction
  source 1..49: mol_type = other DNA
aattctaatacgactcactatagggacagtggaagcaaaataaacacca

SEQ ID NO: 35 - DNA, 37 bp, synthetic construct
  misc_feature 1..37: note = > E.coli 23S rRNA SMART-first probe
  source 1..37: mol_type = other DNA
tctgaatggaaggaccatcgctcaacggattcgaaat

SEQ ID NO: 36 - DNA, 105 bp, synthetic construct
  misc_feature 1..105: note = > E.coli 23S rRNA SMART-Mango second probe
  misc_feature 75: note = /note="n = iSp18"
  misc_feature 105: note = /note="n=3amo"
  source 1..105: mol_type = other DNA
ggcacgtacgaatataccacataccaaaccttccttcgtacgtgccccctatagtgagtcgtattaatttcgaantaaaaggtactccggggataacaggctgan

SEQ ID NO: 37 - RNA, 256 nt, synthetic construct
  misc_feature 1..256: note = > Reverse Complement RNA sequence of E.coli 23S rRNA, NASBAproduct (256-nt)
  source 1..256: mol_type = other RNA
gggacagctcgcgtaccactttaaatggcgaacagccatacccttgggacctacttcagccccaggatgtgatgagccgacatcgaggtgccaaacaccgccgtcgatatgaactcttgggcggtatcagcctgttatccccggagtaccttttatccgttgagcgatggtccttccattcagaaccaccggatcactatgacctgctttcgcacctgctcgcgccgtcacgctcgcagtcaagctggcttatgcc

SEQ ID NO: 38 - RNA, 2904 nt, synthetic construct
  misc_feature 1..2904: note = > NR_103073.1 Escherichia coli strain K-12 23S ribosomal RNAgene, complete sequence
  source 1..2904: mol_type = other RNA
ggttaagcgactaagcgtacacggtggatgccctggcagtcagaggcgatgaaggacgtgctaatctgcgataagcgtcggtaaggtgatatgaaccgttataaccggcgatttccgaatggggaaacccagtgtgtttcgacacactatcattaactgaatccataggttaatgaggcgaaccgggggaactgaaacatctaagtaccccgaggaaaagaaatcaaccgagattcccccagtagcggcgagcgaacggggaggagcccagagcctgaatcagtgtgtgtgttagtggaagcgtctggaaaggcgcgcgatacagggtgacagccccgtacacaaaaatgcacatgctgtgagctcgatgagtagggcgggacacgtggtatcctgtctgaatatggggggaccatcctccaaggctaaatactcctgactgaccgatagtgaaccagtaccgtgagggaaaggcgaaaagaaccccggcgaggggagtgaaaaagaacctgaaaccgtgtacgtacaagcagtgggagcatgcttaggcgtgtgactgcgtaccttttgtataatgggtcagcgacttatattctgtagcaaggttaaccgaataggggagccgaagggaaaccgagtcttaactgggcgttaagttgcagggtatagacccgaaacccggtgatctagccatgggcaggttgaaggttgggtaacactaactggaggaccgaaccgactaatgttgaaaaattagcggatgacttgtggctgggggtgaaaggccaatcaaaccgggagatagctggttctccccgaaagctatttaggtagcgcctcgtgaactcatctccgggggtagagcactgtttcggcaagggggtcatcccgacttaccaacccgatgcaaactgcgaataccggagaatgttatcacgggagacacacggcgggtgctaacgtccgtcgtgaagagggaaacaacccagaccgccagctaaggtcccaaagtcatggttaagtgggaaacgatgtgggaaggcccagacagccaggatgttggcttagaagcagccatcatttaaagaaagcgtaatagctcactggtcgagtcggcctgcgcggaagatgtaacggggctaaaccatgcaccgaagctgcggcagcgacgcttatgcgttgttgggtaggggagcgttctgtaagcctgtgaaggtgtactgtgaggtatgctggaggtatcagaagtgcgaatgctgacataagtaacgataaagcgggtgaaaagcccgctcgccggaagaccaagggttcctgtccaacgttaatcggggcagggtgagtcgacccctaaggcgaggccgaaaggcgtagtcgatgggaaacaggttaatattcctgtacttggtgttactgcgaaggggggacggagaaggctatgttggccgggcgacggttgtcccggtttaagcgtgtaggctggttttccaggcaaatccggaaaatcaaggctgaggcgtgatgacgaggcactacggtgctgaagcaacaaatgccctgcttccaggaaaagcctctaagcatcaggtaacatcaaatcgtaccccaaaccgacacaggtggtcaggtagagaataccaaggcgcttgagagaactcgggtgaaggaactaggcaaaatggtgccgtaacttcgggagaaggcacgctgatatgtaggtgaagcgacttgctcgtggagctgaaatcagtcgaagataccagctggctgcaactgtttattaaaaacacagcactgtgcaaacacgaaagtggacgtatacggtgtgacgcctgcccggtgccggaaggttaattgatggggttagcgcaagcgaagctcttgatcgaagccccggtaaacggcggccgtaactataacggtcctaaggtagcgaaattccttgtcgggtaagttccgacctgcacgaatggcgtaatgatggccaggctgtctccacccgagactcagtgaaattgaactcgctgtgaagatgcagtgtacccgcggcaagacggaaagaccccgtgaacctttactatagcttgacactgaacattgagccttgatgtgtaggataggtgggaggctttgaagtgtggacgccagtctgcatggagccgaccttgaaataccaccctttaatgtttgatgttctaacgttgacccgtaatccgggttgcggacagtgtctggtgggtagtttgactggggcggtctcctcctaaagagtaacggaggagcacgaaggttggctaatcctggtcggacatcaggaggttagtgcaatggcataagccagcttgactgcgagcgtgacggcgcgagcaggtgcgaaagcaggtcatagtgatccggtggttctgaatggaagggccatcgctcaacggataaaaggtactccggggataacaggctgataccgcccaagagttcatatcgacggcggtgtttggcacctcgatgtcggctcatcacatcctggggctgaagtaggtcccaagggtatggctgttcgccatttaaagtggtacgcgagctgggtttagaacgtcgtgagacagttcggtccctatctgccgtgggcgctggagaactgaggggggctgctcctagtacgagaggaccggagtggacgcatcactggtgttcgggttgtcatgccaatggcactgcccggtagctaaatgcggaagagataagtgctgaaagcatctaagcacgaaacttgccccgagatgagttctccctgactccttgagagtcctgaaggaacgttgaagacgacgacgttgataggccgggtgtgtaagcgcagcgatgcgttgagctaaccggtactaatgaaccgtgaggcttaacctt

SEQ ID NO: 39 - RNA, 79 nt, synthetic construct
  misc_feature 1..79: note = > Synthetic RNA target of 23S ribosomal RNA (79-nt, pos.2393-2468, reverse complement)
  source 1..79: mol_type = other RNA
gggagggcggtatcagcctgttatccccggagtaccttttatccgttgagcgatggtccttccattcagaaccaccgga

SEQ ID NO: 40 - DNA, 38 bp, synthetic construct
  misc_feature 1..38: note = > S.aureus mecA SMART-first probe
  source 1..38: mol_type = other DNA
aggtgaaatactgattaacccagtacagatttcgaaat

SEQ ID NO: 41 - DNA, 106 bp, synthetic construct
  misc_feature 1..106: note = > S.aureus mecA SMART-Mango second probe
  misc_feature 75: note = /note="n = iSp18"
  misc_feature 106: note = /note="n=3amo"
  source 1..106: mol_type = other DNA
ggcacgtacgaatataccacataccaaaccttccttcgtacgtgccccctatagtgagtcgtattaatttcgaancctttcaatctatagcgcattagaaaataan

SEQ ID NO: 42 - RNA, 98 nt, synthetic construct
  misc_feature 1..98: note = > Reverse Complement RNA sequence of S.aureus mecA gene, NASBAproduct (98-nt)
  source 1..98: mol_type = other RNA
gggaagtgaggtgcgttaatattgccattattttctaatgcgctatagattgaaaggatctgtactgggttaatcagtatttcaccttgtccgtaacc

SEQ ID NO: 43 - DNA, 475 bp, synthetic construct
  misc_feature 1..475: note = >KX639010.1 Staphylococcus aureus strain SQ5 methicillinresistance protein subunit A (mecA) gene, partial cds
  source 1..475: mol_type = other DNA
tgtaaaggttggcaaaaagataaatcttggggtggttacaacgttacaagatatgaagtggtaaatggtaatatcgacttaaaacaagggatagaatcatcagataacattttctttgctagagtagcactcgaattaggcagtaagaaatttgaaaaaggcatgaaaaaactaggtgttggtgaagatataccaagccattatccattttatagggctcaaatttcaaacaaaaatttagataatgaaatattattagctgattcaggttacggacaaggtgaaatactgattaacccagtacagatcctttcaatctatagcgcattagaaggtaatggcaatattaacgcacctcacttattaaaagacacgaaaaacaaagtttggaagaaaaatattatttccaaagaaaatatcaatctattaactgatggtatgcaacaagtcgtaaataaaacacataaagaagata

SEQ ID NO: 44 - RNA, 98 nt, synthetic construct; identical to SEQ ID NO: 42
  misc_feature 1..98: note = > Synthetic RNA target of S.aureus mecA RNA (98-nt, pos. 268-362,reverse complement)
  source 1..98: mol_type = other RNA

SEQ ID NO: 45 - DNA, 23 bp, synthetic construct
  misc_feature 1..23: note = > Influenza A PB1 gene SMART-first probe (15-nt targethybridization region)
  source 1..23: mol_type = other DNA
ggctgtatggaggatttcgaaat

SEQ ID NO: 46 - DNA, 23 bp, synthetic construct
  misc_feature 1..23: note = > Influenza B PA gene SMART-first probe (15-nt targethybridization region)
  source 1..23: mol_type = other DNA
ccatccatgctatggttcgaaat

SEQ ID NO: 47 - DNA, 91 bp, synthetic construct
  misc_feature 1..91: note = > Influenza A PB1 gene SMART-second probe (15-nt targethybridization region)
  misc_feature 75: note = /note="n = iSp18"
  misc_feature 91: note = /note="n=3amo"
  source 1..91: mol_type = other DNA
ggcacgtacgaatataccacataccaaaccttccttcgtacgtgccccctatagtgagtcgtattaatttcgaanctccagtataagggan

SEQ ID NO: 48 - DNA, 91 bp, synthetic construct
  misc_feature 1..91: note = > Influenza B PA gene SMART-second probe (15-nt targethybridization region)
  misc_feature 75: note = /note="n = iSp18"
  misc_feature 91: note = /note="n=3amo"
  source 1..91: mol_type = other DNA
ggcacgtacgaatataccacataccaaaccttccttcgtacgtgccccctatagtgagtcgtattaatttcgaanttcttggcattccctn

SEQ ID NO: 49 - RNA, 30 nt, synthetic construct
  misc_feature 1..30: note = > Synthetic RNA target of Influenza A PB1 gene (30-nt)
  source 1..30: mol_type = other RNA
tcccttatactggagatcctccatacagcc

SEQ ID NO: 50 - RNA, 30 nt, synthetic construct
  misc_feature 1..30: note = > Synthetic RNA target of Influenza B PA gene (30-nt)
  source 1..30: mol_type = other RNA
agggaatgccaagaaccatagcatggatgg

SEQ ID NO: 51 - DNA, 2274 bp, synthetic construct
  misc_feature 1..2274: note = >MK185298.1 Influenza A virus (A/swine/SouthDakota/A02016893/2018(H1N1)) segment 2 polymerase PB1 (PB1) andPB1-F2 protein (PB1-F2) genes, complete cds
  source 1..2274: mol_type = other DNA
atggatgtcaatccgactctacttttcctaaaggttccagcgcaaaatgccataagcaccacattcccttatactggagatcctccatacagccatggaacaggaacaggatacactatggacacagtcaacagaacacaccaatattcagaaaaagggaaatggacaacaaacacagaaactggggcaccccagctcaacccgattgatggaccactacctgaagataatgaaccaagtggatatgcacaaacagactgtgtcctggaggccatggctttccttgaggaatcccacccagggatatttgagaattcatgccttgaaacaatggaaattgtccaacaaacaagggtggataaattaactcaaggtcgtcagacttatgattggacattgaacagaaaccagccggcagcaactgcattggccaacaccatagaagtttttagatcaaacgggctaacggctaatgagtcaggaaggctaatagatttcctaaaagatgtaatggaatcaatggataaagaggaaatagagataacaacacactttcaaagaaaaaggagagtaagagacaacatgaccaaaaagatggtaacacaaagaacaatagggaagaaaaaacaaagaatgagtaagaaaagttatctaataagggcactaacattaaatacgatgaccaaagatgcagagagaggcaagttaaaaaggagggctatcgcaacacctgggatgcaaattagagggttcgtgtactttgttgaaactttagctagaagcatttgcgaaaagcttgaacagtccggactcccagtagggggcaatgaaaagaaagccaaattggcaaatgttgtgagaaagatgatgactaattcacaagacacagagctttctttcacaatcactggagacaacactaagtggaatgagaaccaaaatccccgaatgttcctggcaatgattacatacatcaccagaaatcaacccgagtggttcagaaacatactgagcatggcaccaataatgttctcaaacaaaatggcaagactaggaaaagggtacatgttcgagagtaaaagaatgaagcttcgaacacaagtaccagcagaaatgttggcaagcattgacctgaagtattttaatgaatcaacacggaagaaaatcgaaaaaataaggcctctcctaatagatggcacagcatcattgagccctgggatgatgatgggcatgttcaacatgctaagtacggttttgggagtctcaatattgaatcttggacagaagaaatacaccaggacaacatattggtgggatggactccaatcctccgacgattttgccctcatagtaaatgcaccaaaccatgagggaatacaagcaggagtggatagattctacaggacctgcaagttagtagggatcaacatgagcaagaagaagtcctacataaataggactggaacatttgaattcacaagctttttttatcgctatgggtttgtagctaattttagcatggagctgcccagttttggagtgtctggaataaacgaatcagctgacatgagtatcggggtaacagttataaagaataacatgataaataatgatcttggacctgcaacagcccagatggcccttcagctattcatcaaagactacagatacacatatagatgccatagaggggacacactaattcagacgagaagatcattcgagctaaagagcctgtgggatcaaacccaatcaaaggcagggttattagtatctgatggaggaccgaatttatacaacatccggaatcttcacattcctgaagtctgcttaaaatgggagctaatggatgaggattatcggggaagactttgcaatcccctaaatccttttgtcagccataaagagatcgattctgtgaacagtgctgttgtgatgccagcccatggtccagccaaaagcatggaatatgatgccgtcgcaactacacactcctggattcccaaaaggaaccgctctattctcaacacgagccaaaggggaattcttgaggatgaacagatgtaccagaagtgctgcaacctgttcgagaaatttttccctagtagttcatacaggagaccggttggaatttctagcatggtggaggccatggtgtctagggcccggattgatgccaggattgacttcgaatctggacggatcaaaaaagaagagttttctgagatcatgaagatctgttccaccattgaagaactcagacggcaaaagtga

SEQ ID NO: 52 - DNA, 2181 bp, synthetic construct
  misc_feature 1..2181: note = >MT637912.1 Influenza B virus (B/Texas/9813/2019) segment 3polymerase PA (PA) gene, complete cds
  source 1..2181: mol_type = other DNA
atggatacctttattacaagaaacttccagactacaataatacaaaaggccaaaaacacaatggcagaatttagtgaagatcctgaattgcaaccagcaatgctattcaacatctgtgtccatctagaggtttgctatgtaataagtgacatgaattttcttgacgaagaaggaaaagcatatacagcattagaaggacaaggaaaagaacaaaatttgagaccacaatatgaagtaattgagggaatgccaagaaccatagcatggatggtccaaagatccttagctcaagagcatgggatagagactcccaagtatctggctgatttgtttgattataagaccaagagatttatagaagttggaataacaaaaggattggctgatgattacttttggaaaaagaaagagaagctgggaaatagcatggaactaatgatattcagctacaatcaagactattcattaagtaatgaatcctcattggatgaggaagggaaagggagagtgctaagcaggctcacagaacttcaagctgaattaagtctgaaaaacttatggcaagttctcataggagaagaagatgttgaaaagggaattgactttagacttggacaaacaatatctagactgagggatatatctgttcctgctggtttctccaattttgaaggaatgaggagctacatagacaatatagacccgaaaggagcaatagagagaaacctagcaaggatgtctcccttagtatcagtcacacctaaaaagttgaaatgggaggatctaagaccaatagggcctcacatttacaaccatgagctaccagaagttccatacaatgcctttcttttaatgtctgatgaactggggctggccaatatgacggagggaaagtccaaaaaaccaaagacattagccaaagaatgtctagaaaagtactcaacactgcgggatcagactgacccaatattaatagtgaaaagcgaaaaagctaacgaaaatttcctatggaaactttggagagactgtgtaaatacaataagcaatgaggaaatgagtaacgagttacagaaaaccaattatgccaagtgggccacaggggatggtttaacataccaaaaaataatgaaagaagtagcaatagatgacgaaacaatgtgccaagaagagcctaaaatccctaacaagtgtagagtggctgcttgggttcaaacagagatgaacctattgagcactctgacaagtaaaagagctctggacctaccagaaatagggccagacgtggcaccagtggagcatgttggaagtgaaagaagaaaatactttgttaatgaaatcaactactgtaaggcctctacagttatgatgaagtatgtgctttttcacacttcattgctgaatgaaagcaatgccagcatgggaaaatacaaagtaataccaataaccaatagaatagtaaatgaaaaaggagaaagtttcgacatgctttatggtctggcagttaaaggacaatctcatctgaggggggacactgatgttgtaacagttgtaactttcgaatttagtagtacagaccccagagtggactcaggaaagtggccgaaatatactgtgtttaggattggctccctatttgtgggtgggagggaaaaatctgtgtacctatattgcagagtgaatggcacaaataagatccaaatgaaatggggaatggaagctagaagatgtctgcttcaatcaatgcaacaaatggaagcaattgttgaacaagaatcctcgatacaaggatacgacatgaccaaagcttgtttcaagggggacagaataaatagccccaaaactttcagtattggaactcaagaagggaaactagtaaaaggatcctttggaaaagcactaagagtaatatttaccaaatgtttgatgcactatgtatttggaaatgcccagttggagggattcagtgccgagtctaggagacttctactgttgattcaagcattaaaggacagaaagggcccttgggtgttcgacttagagggaatgtactctggaatagaagaatgtatcagtaacaacccttgggtaatacagagtgcatactggttcaatgaatggttgggttttgaaaaggagggaagtaaagtattagaatcagtagatgaaataatggatgaataa

SEQ ID NO: 53 - DNA, 20 bp, synthetic construct
  misc_feature 1..20: note = > 5 primer for E.coli 23S rRNA NASBA amplification reaction
  source 1..20: mol_type = other DNA
ggcataagccagcttgactg

SEQ ID NO: 54 - DNA, 46 bp, synthetic construct
  misc_feature 1..46: note = > 3 primer for E.coli 23S rRNA NASBA amplification reaction
  source 1..46: mol_type = other DNA
aattctaatacgactcactatagggacagctcgcgtaccactttaa

SEQ ID NO: 55 - DNA, 20 bp, synthetic construct
  misc_feature 1..20: note = > 5 primer for S.aureus mecA+ NASBA amplification reaction
  source 1..20: mol_type = other DNA
ggttacggacaaggtgaaat

SEQ ID NO: 56 - DNA, 46 bp, synthetic construct
  misc_feature 1..46: note = > 3 primer for S.aureus mecA+ NASBA amplification reaction
  source 1..46: mol_type = other DNA
aattctaatacgactcactatagggaagtgaggtgcgttaatattg

SEQ ID NO: 57 - RNA, 49 nt, synthetic construct
  misc_feature 1..49: note = > Broccoli RNA aptamer (49-nt, Filonov et al. JACS, 2014)
  source 1..49: mol_type = other RNA
gagacggtcgggtccagatattcgtatctgtcgagtagagtgtgggctc

SEQ ID NO: 58 - DNA, 108 bp, synthetic construct
  misc_feature 1..108: note = > E.coli 16S rRNA SMART-Broccoli second probe
  misc_feature 78: note = /note="n = iSp18"
  misc_feature 108: note = /note="n=3amo"
  source 1..108: mol_type = other DNA
gagcccacactctactcgacagatacgaatatctggacccgaccgtctcccctatagtgagtcgtattaatttcgaanggccttcgggttgtaaagtactttcagcgn

SEQ ID NO: 59 - DNA, 109 bp, synthetic construct
  misc_feature 1..109: note = > SARS-CoV-2 T3 SMART-Broccoli second probe
  misc_feature 78: note = /note="n = iSp18"
  misc_feature 109: note = /note="n=3amo"
  source 1..109: mol_type = other DNA
gagcccacactctactcgacagatacgaatatctggacccgaccgtctcccctatagtgagtcgtattaatttcgaancaatggtactaagaggtttgataaccctgtn

SEQ ID NO: 60 - DNA, 46 bp, synthetic construct
  misc_feature 1..46: note = > Mango aptamer (Reverse Complement)
  source 1..46: mol_type = other DNA
ggcacgtacgaatataccacataccaaaccttccttcgtacgtgcc

SEQ ID NO: 61 - DNA, 49 bp, synthetic construct
  misc_feature 1..49: note = > Broccoli aptamer (Reverse Complement)
  source 1..49: mol_type = other DNA
gagcccacactctactcgacagatacgaatatctggacccgaccgtctc

SEQ ID NO: 62 - DNA, 17 bp, synthetic construct
  misc_feature 1..17: note = > T7 Promoter (Reverse Complement)
  source 1..17: mol_type = other DNA
tatagtgagtcgtatta

SEQ ID NO: 63 - DNA, 101 bp, synthetic construct
  misc_feature 1..101: note = similar to SEQ ID NO: 2, but substituting iSp18 for any spacerand optionally including any blocker molecule at the 3 end
  misc_feature 75: note = /note="n = iSp18"
  source 1..101: mol_type = other DNA
ggcacgtacgaatataccacataccaaaccttccttcgtacgtgccccctatagtgagtcgtattaatttcgaanggcatgacaacccgaacaccagtgat

SEQ ID NO: 64 - DNA, 104 bp, synthetic construct
  misc_feature 1..104: note = similar to SEQ ID NO: 8, but substituting iSp18 for any spacerand optionally including any blocker molecule at the 3 end
  misc_feature 75: note = /note="n = iSp18"
  source 1..104: mol_type = other DNA
ggcacgtacgaatataccacataccaaaccttccttcgtacgtgccccctatagtgagtcgtattaatttcgaanggccttcgggttgtaaagtactttcagcg

SEQ ID NO: 65 - DNA, 97 bp, synthetic construct
  misc_feature 1..97: note = similar to SEQ ID NO: 23, but substituting iSp18 for any spacerand optionally including any blocker molecule at the 3 end
  misc_feature 75: note = /note="n = iSp18"
  source 1..97: mol_type = other DNA
ggcacgtacgaatataccacataccaaaccttccttcgtacgtgccccctatagtgagtcgtattaatttcgaanggccttcgggttgtaaagtact

SEQ ID NO: 66 - DNA, 90 bp, synthetic construct
  misc_feature 1..90: note = similar to SEQ ID NO: 24, but substituting iSp18 for any spacerand optionally including any blocker molecule at the 3 end
  misc_feature 75: note = /note="n = iSp18"
  source 1..90: mol_type = other DNA
ggcacgtacgaatataccacataccaaaccttccttcgtacgtgccccctatagtgagtcgtattaatttcgaanggccttcgggttgta

SEQ ID NO: 67 - DNA, 82 bp, synthetic construct
  misc_feature 1..82: note = similar to SEQ ID NO 25, but substituting iSp18 for any spacerand optionally including any blocker molecule at the 3 end
  misc_feature 75: note = /note="n = iSp18"
  source 1..82: mol_type = other DNA
ggcacgtacgaatataccacataccaaaccttccttcgtacgtgccccctatagtgagtcgtattaatttcgaanggccttc

SEQ ID NO: 68 - DNA, 105 bp, synthetic construct
  misc_feature 1..105: note = similar to SEQ ID NO 27, but substituting iSp18 for any spacerand optionally including any blocker molecule at the 3 end
  misc_feature 75: note = /note="n = iSp18"
  source 1..105: mol_type = other DNA
ggcacgtacgaatataccacataccaaaccttccttcgtacgtgccccctatagtgagtcgtattaatttcgaancaatggtactaagaggtttgataaccctgt

SEQ ID NO: 69 - DNA, 104 bp, synthetic construct
  misc_feature 1..104: note = similar to SEQ ID NO: 36, but substituting iSp18 for any spacerand optionally including any blocker molecule at the 3 end
  misc_feature 75: note = /note="n = iSp18"
  source 1..104: mol_type = other DNA
ggcacgtacgaatataccacataccaaaccttccttcgtacgtgccccctatagtgagtcgtattaatttcgaantaaaaggtactccggggataacaggctga

SEQ ID NO: 70 - DNA, 105 bp, synthetic construct
  misc_feature 1..105: note = similar to SEQ ID NO: 41, but substituting iSp18 for any spacerand optionally including any blocker molecule at the 3 end
  misc_feature 75: note = /note="n = iSp18"
  source 1..105: mol_type = other DNA
ggcacgtacgaatataccacataccaaaccttccttcgtacgtgccccctatagtgagtcgtattaatttcgaancctttcaatctatagcgcattagaaaataa

SEQ ID NO: 71 - DNA, 90 bp, synthetic construct
  misc_feature 1..90: note = similar to SEQ ID NO: 47, but substituting iSp18 for any spacerand optionally including any blocker molecule at the 3 end
  misc_feature 75: note = /note="n = iSp18"
  source 1..90: mol_type = other DNA
ggcacgtacgaatataccacataccaaaccttccttcgtacgtgccccctatagtgagtcgtattaatttcgaanctccagtataaggga

SEQ ID NO: 72 - DNA, 90 bp, synthetic construct
  misc_feature 1..90: note = similar to SEQ ID NO: 48, but substituting iSp18 for any spacerand optionally including any blocker molecule at the 3 end
  misc_feature 75: note = /note="n = iSp18"
  source 1..90: mol_type = other DNA
ggcacgtacgaatataccacataccaaaccttccttcgtacgtgccccctatagtgagtcgtattaatttcgaanttcttggcattccct

SEQ ID NO: 73 - DNA, 107 bp, synthetic construct
  misc_feature 1..107: note = similar to SEQ ID NO: 58, but substituting iSp18 for any spacerand optionally including any blocker molecule at the 3 end
  misc_feature 78: note = /note="n = iSp18"
  source 1..107: mol_type = other DNA
gagcccacactctactcgacagatacgaatatctggacccgaccgtctcccctatagtgagtcgtattaatttcgaanggccttcgggttgtaaagtactttcagcg

SEQ ID NO: 74 - DNA, 108 bp, synthetic construct
  misc_feature 1..108: note = similar to SEQ ID NO: 59, but substituting iSp18 for any spacerand optionally including any blocker molecule at the 3 end
  misc_feature 78: note = /note="n = iSp18"
  source 1..108: mol_type = other DNA
gagcccacactctactcgacagatacgaatatctggacccgaccgtctcccctatagtgagtcgtattaatttcgaancaatggtactaagaggtttgataaccctgt

SEQ ID NO: 75 - DNA, 26 bp, synthetic construct
  source 1..26: mol_type = other DNA
  misc_feature 1..26: note = Fig. 4 first portion of target RNA
aatggcactgcccggtagctaaatgc

SEQ ID NO: 76 - DNA, 26 bp, synthetic construct
  source 1..26: mol_type = other DNA; note = Fig. 4 second portion of target RNA
atcactggtgttcgggttgtcatgcc